European Patent Application EP 4 389 770 A1, published June 26, 2024. Title: Bispecific antibody and use thereof. Applicant: BIOTHEUS INC. The sequence listing filed with the application follows.

SEQUENCE LISTING (29 sequences)

SEQ ID NO: 1 - protein, 119 aa, synthetic construct
QVQLVQSGAEVKKPGASVKVSCKASGYTFTSYYMHWVRQAPGQGLEWMGTIYPGNGDTSYNQKFQGRVTMTRDKSTSTVYMELSSLRSEDTAVYFCARGGYYGNSLDYWGQGTLVTVSS

SEQ ID NO: 2 - protein, 113 aa, synthetic construct
DIVMTQSPDSLAVSLGERATINCKSSQSVLSSGNQKNYLAWYQQKPGQPPKLLIYWASTRESGVPDRFSGSGSGTDFTLTISSLQAEDVAVYYCQNAYYYPFTFGQGTKLEIK

SEQ ID NO: 3 - protein, 125 aa, synthetic construct
QVQLVESGGGVVQPGRSLRLSCAASGSTFSIVAMGWYRQAPGKQRELVASIITGDGDTNYADSVKGRFTISRDNSKNTMYLQMNSLKPEDTAVYYCYARTGEGSSWLEGHEYDYWGQGTQVTVSS

SEQ ID NO: 4 - protein, 330 aa, synthetic construct
ASTKGPSVFPLAPSSKSTSGGTAALGCLVKDYFPEPVTVSWNSGALTSGVHTFPAVLQSSGLYSLSSVVTVPSSSLGTQTYICNVNHKPSNTKVDKKVEPKSCDKTHTCPPCPAPEAAGGPSVFLFPPKPKDTLMISRTPEVTCVVVDVSHEDPEVKFNWYVDGVEVHNAKTKPREEQYNSTYRVVSVLTVLHQDWLNGKEYKCKVSNKALPAPIEKTISKAKGQPREPQVYTLPPSREEMTKNQVSLTCLVKGFYPSDIAVEWESNGQPENNYKTTPPVLDSDGSFFLYSKLTVDKSRWQQGNVFSCSVMHEALHNHYTQKSLSLSPGK

SEQ ID NO: 5 - protein, 20 aa, synthetic construct
GGGGSGGGGSGGGGSGGGGS

SEQ ID NO: 6 - protein, 594 aa, synthetic construct
QVQLVQSGAEVKKPGASVKVSCKASGYTFTSYYMHWVRQAPGQGLEWMGTIYPGNGDTSYNQKFQGRVTMTRDKSTSTVYMELSSLRSEDTAVYFCARGGYYGNSLDYWGQGTLVTVSSASTKGPSVFPLAPSSKSTSGGTAALGCLVKDYFPEPVTVSWNSGALTSGVHTFPAVLQSSGLYSLSSVVTVPSSSLGTQTYICNVNHKPSNTKVDKKVEPKSCDKTHTCPPCPAPEAAGGPSVFLFPPKPKDTLMISRTPEVTCVVVDVSHEDPEVKFNWYVDGVEVHNAKTKPREEQYNSTYRVVSVLTVLHQDWLNGKEYKCKVSNKALPAPIEKTISKAKGQPREPQVYTLPPSREEMTKNQVSLTCLVKGFYPSDIAVEWESNGQPENNYKTTPPVLDSDGSFFLYSKLTVDKSRWQQGNVFSCSVMHEALHNHYTQKSLSLSPGKGGGGSGGGGSGGGGSGGGGSQVQLVESGGGVVQPGRSLRLSCAASGSTFSIVAMGWYRQAPGKQRELVASIITGDGDTNYADSVKGRFTISRDNSKNTMYLQMNSLKPEDTAVYYCYARTGEGSSWLEGHEYDYWGQGTQVTVSS

SEQ ID NO: 7 - protein, 220 aa, synthetic construct
DIVMTQSPDSLAVSLGERATINCKSSQSVLSSGNQKNYLAWYQQKPGQPPKLLIYWASTRESGVPDRFSGSGSGTDFTLTISSLQAEDVAVYYCQNAYYYPFTFGQGTKLEIKRTVAAPSVFIFPPSDEQLKSGTASVVCLLNNFYPREAKVQWKVDNALQSGNSQESVTEQDSKDSTYSLSSTLTLSKADYEKHKVYACEVTHQGLSSPVTKSFNRGEC

SEQ ID NO: 8 - protein, 107 aa, synthetic construct [sequence omitted]

SEQ ID NO: 9 - protein, 8 aa, synthetic construct
GYTFTSYY

SEQ ID NO: 10 - protein, 8 aa, synthetic construct
IYPGNGDT

SEQ ID NO: 11 - protein, 12 aa, synthetic construct
ARGGYYGNSLDY

SEQ ID NO: 12 - protein, 12 aa, synthetic construct
QSVLSSGNQKNY

SEQ ID NO: 13 - skipped

SEQ ID NO: 14 - protein, 9 aa, synthetic construct
QNAYYYPFT

SEQ ID NO: 15 - protein, 8 aa, synthetic construct
GSTFSIVA

SEQ ID NO: 16 - protein, 8 aa, synthetic construct
IITGDGDT

SEQ ID NO: 17 - protein, 18 aa, synthetic construct
YARTGEGSSWLEGHEYDY

SEQ ID NO: 18 - DNA, 1782 bp, synthetic construct
  source 1..1782: mol_type = other DNA
caggtgcagctggttcagtctggcgccgaagtgaagaaacctggcgcctctgtgaaggtgtcctgcaaggcttccggctacacctttaccagctactacatgcactgggtccgacaggcccctggacaaggattggagtggatgggcaccatctatcccggcaacggcgacacctcctacaaccagaaattccagggcagagtgaccatgaccagagacaagtccacctccaccgtgtacatggaactgtccagcctgagatccgaggataccgccgtgtacttctgtgccagaggcggctactacggcaactccctggattattggggccagggcacactggtcaccgtgtcctctgcttctaccaagggacccagcgtgttccctctggctccttccagcaagtctacctctggcggaacagctgctctgggctgcctcgtgaaggactactttcctgagcctgtgaccgtgtcttggaactctggcgctctgacatccggcgtgcacacatttccagctgtgctgcagtcctccggcctgtactctctgtcctctgtcgtgaccgtgccttccagctctctgggaacccagacctacatctgcaatgtgaaccacaagccttccaacaccaaggtggacaagaaggtggaacccaagtcctgcgacaagacccacacctgtcctccatgtcctgctccagaagctgctggcggcccttccgtgtttctgttccctccaaagcctaaggacaccctgatgatctctcggacccctgaagtgacctgcgtggtggtggatgtgtctcacgaggacccagaagtgaagttcaattggtacgtggacggcgtggaagtgcacaacgccaagaccaagcctagagaggaacagtacaactccacctacagagtggtgtccgtgctgaccgtgctgcaccaggattggctgaacggcaaagagtacaagtgcaaggtgtccaacaaggccctgcctgctcctatcgaaaagaccatctccaaggccaagggccagcctcgagaaccccaggtttacaccctgcctccaagccgggaagagatgaccaagaaccaggtgtccctgacctgcctggtcaagggcttctacccttccgacattgccgtggaatgggagagcaatggccagccagagaacaactacaagacaacccctcctgtgctggactccgacggctcattcttcctgtactccaagctgacagtggacaagtcccggtggcagcagggcaacgtgttctcctgttctgtgatgcacgaggccctgcacaaccactacacacagaagtccctgtctctgtcccctggcaaaggtggcggaggatctggcggaggtggaagcggcggaggcggttctggtggtggcggatctcaagttcagctggtggaatctggcggcggagtggttcagcctggaagatccctgagactgtcttgcgccgcttctggctccaccttcagcatcgttgccatgggctggtacagacaggctcctggcaaacagcgagagctggtggcctctatcattaccggcgacggcgataccaactacgccgactctgtgaaaggccggttcaccatctctcgggacaactccaagaacaccatgtacctgcagatgaactccctgaagcctgaggatacagctgtctactactgctacgccagaaccggcgagggatcctcttggctggagggccacgagtacgactactggggacagggaacacaagtgacagtgtcctcc

SEQ ID NO: 19 - DNA, 660 bp, synthetic construct
  source 1..660: mol_type = other DNA
gacatcgtgatgacccagtctccagactctctggccgtgtctctgggcgagagagccaccatcaactgcaagtcctctcagtccgtgctgtcctccggcaaccagaagaattacctggcctggtatcagcagaagcccggccagcctcctaagctgctgatctactgggcctccaccagagaatctggcgtgcccgatagattctccggctctggctctggcaccgactttaccctgacaatcagctccctgcaggccgaggatgtggccgtgtactactgtcagaacgcctactactaccccttcaccttcggccagggcaccaagctggaaatcaagagaaccgtggccgctccttccgtgttcatcttcccaccttccgacgagcagctgaagtccggcacagcttctgtcgtgtgcctgctgaacaacttctaccctcgggaagccaaggtgcagtggaaggtggacaatgccctgcagtccggcaactcccaagagtctgtgaccgagcaggactctaaggactccacctacagcctgtcctccacactgaccctgtccaaggccgactacgagaagcacaaggtgtacgcctgcgaagtgacccatcagggcctgtctagccctgtgaccaagtctttcaaccggggcgagtgt

SEQ ID NO: 20 - DNA, 1341 bp, synthetic construct
  source 1..1341: mol_type = other DNA
caggtccagctgcagcagtggggcgccggactgctgaagccaagcgaaacactgagcctgacctgcgccgtctacggaggatccttttcaggatactattggagctggatcagacagtcccccgaaaagggcctggagtggatcggagagattaaccacggaggatacgtgacctacaaccccagcctggagagcagagtgaccatcagtgtggacacctcaaagaaccagtttagcctgaaactgagcagcgtgaccgccgccgacaccgcagtctactactgcgctagagactacggcccaggcaactacgactggtacttcgacctgtggggcagaggcaccctggtgacagtgagcagcgccagcaccaagggccctagcgtgtttcccctggccccttgttccagaagcacatccgagtccaccgccgccctgggctgtctggtgaaggattactttcccgagcccgtgacagtgtcctggaacagcggcgccctgacatccggcgtgcacaccttccccgccgtgctgcagtcctccggcctgtacagcctgagcagcgtggtgaccgtgcccagcagcagcctgggcaccaagacatacacctgtaacgtggatcacaagcccagcaacaccaaggtggataagagggtggagagcaagtacggccccccttgccccccctgccctgctcctgagttcctgggcggccccagcgtgttcctgttcccccctaagcccaaggacacactgatgatctccagaacccccgaggtgacctgtgtggtggtggacgtgagccaggaggaccctgaggtgcagtttaactggtacgtggacggcgtggaggtgcacaatgccaagacaaagcctcgggaggagcagttcaactccacatacagagtggtgtccgtgctgacagtgctgcaccaggactggctgaacggcaaggagtacaagtgtaaggtgagcaacaagggcctgcccagcagcatcgagaagaccatctccaaggccaagggccagcccagggagcctcaggtgtacacactgcctcctagccaggaggagatgaccaagaaccaggtgagcctgacctgcctggtgaagggcttctacccttccgatattgccgtggagtgggagtccaatggccagcccgagaataactacaagacaacccctcctgtgctggattccgacggctcctttttcctgtacagcaggctgacagtggataagagcaggtggcaggagggcaacgtgttcagctgtagcgtgatgcacgaggccctgcacaaccactacacccagaagagcctgtccctgtccctgggc

SEQ ID NO: 21 - DNA, 648 bp, synthetic construct
  source 1..648: mol_type = other DNA
gagattgtgctgacccagagccccgccacactgagtctgagtcccggcgagagagcaacactgagttgtagggcaagccagagcgtgagtagctacctggcctggtaccagcagaagcccggccaggcccccagactgctgatttacgacgcctccaacagagcaaccggaatccccgccagattcagcggaagcggcagcggcaccgacttcaccctgactatcagcagcctggaacccgaggatttcgccgtctactactgccagcagcgcagcaactggccccccgctctgaccttcggaggaggcacaaaggtggaaatcaagcgaactgtggctgcaccatctgtcttcatcttcccgccatctgatgagcagttgaaatctggaactgcctctgttgtgtgcctgctgaataacttctatcccagagaggccaaagtacagtggaaggtggataacgccctccaatcgggtaactcccaggagagtgtcacagagcaggacagcaaggacagcacctacagcctcagcagcaccctgacgctgagcaaagcagactacgagaaacacaaagtctacgcctgcgaagtcacccatcagggcctgagctcgcccgtcacaaagagcttcaacaggggagagtgc

SEQ ID NO: 22 - DNA, 1056 bp, synthetic construct
  source 1..1056: mol_type = other DNA
caggtgcagctggttgaatctggtggcggagtggtgcagcctggcagatctctgagactgtcttgtgccgcctccggctccaccttttctatcgtggctatgggctggtacagacaggcccctggcaaacagagagagctggtcgcctctatcattaccggcgacggcgataccaactacgccgactctgtgaagggcagattcaccatcagccgggacaactccaagaacaccatgtacctgcagatgaactccctgaagcctgaggacaccgccgtgtactactgctacgctagaaccggcgagggctcctcttggctggaaggccacgagtacgattattggggccagggcacccaagtgaccgtgtcctctgacaagacccacacctgtcctccatgtcctgctccagaagctgctggcggcccttccgtgtttctgttccctccaaagcctaaggataccctgatgatctctcggacccctgaagtgacctgcgtggtggtggatgtgtctcacgaggatcccgaagtgaagttcaattggtacgtggacggcgtggaagtgcacaacgccaagaccaagcctagagaggaacagtacaactccacctacagagtggtgtccgtgctgaccgtgctgcaccaggattggctgaacggcaaagagtacaagtgcaaggtgtccaacaaggccctgcctgctcctatcgaaaagaccatctccaaggccaagggccagcctcgagaaccccaggtttacaccctgcctccaagccgggaagagatgaccaagaaccaggtgtccctgacctgcctcgtgaagggcttctacccttccgacattgccgtggaatgggagagcaatggccagccagagaacaactacaagacaacccctcctgtgctggactccgacggctcattcttcctgtactccaagctgacagtggacaagtccagatggcagcagggcaacgtgttctcctgctccgtgatgcacgaggccctgcacaatcactacacccagaagtccctgtctctgagccctggcaag

SEQ ID NO: 23 - DNA, 1347 bp, synthetic construct
  source 1..1347: mol_type = other DNA
caggtgcagctggtgcagagcggcgccgaggtgaaaaagcccggcgccagcgtgaaggtgagctgcaaggccagcggctacaccttcaccagctactacatgcactgggtgagacaggcccccggccagggcctggagtggatgggcaccatctaccccggcaacggcgacaccagctacaaccagaagttccagggcagagtgaccatgaccagagacaagagcaccagcaccgtgtacatggagctgagcagcctgagaagcgaggacaccgccgtgtacttctgcgccagaggcggctactacggcaacagcctggactactggggccagggcaccctggtgaccgtgagcagcgctagcaccaagggcccatcggtcttccccctggcaccctcctccaagagcacctctgggggcacagcggccctgggctgcctggtcaaggactacttccccgaaccggtgacggtgtcgtggaactcaggcgccctgaccagcggcgtgcacaccttcccggctgtcctacagtcctcaggactctactccctcagcagcgtggtgaccgtgccctccagcagcttgggcacccagacctacatctgcaacgtgaatcacaagcccagcaacaccaaggtggacaagaaagttgagcccaaatcttgtgacaaaactcacacatgcccaccgtgcccagcacctgaactcctggggggaccgtcagtcttcctcttccccccaaaacccaaggacaccctcatgatctcccggacccccgaggtcacatgcgtggtggtggacgtgagccacgaagaccctgaggtcaagttcaactggtacgtggacggcgtggaggtgcataatgccaagacaaagccgcgggaggagcagtacaacagcacgtaccgtgtggtcagcgtcctcaccgtcctgcaccaggactggctgaatggcaaggagtacaagtgcaaggtctccaacaaagccctcccagcccccatcgagaaaaccatctccaaagccaaagggcagccccgagaaccacaggtgtacaccctgcccccatcccgggacgagctgaccaagaaccaggtcagcctgacctgcctggtcaaaggcttctatcccagcgacatcgccgtggagtgggagagcaatgggcagccggagaacaactacaagaccacgcctcccgtgctggactccgacggctccttcttcctctacagcaagctcaccgtggacaagagcaggtggcagcaggggaacgtcttctcatgctccgtgatgcatgaggctctgcacaaccactacacgcagaagagcctctccctgtctccgggtaaa

SEQ ID NO: 24 - DNA, 660 bp, synthetic construct
  source 1..660: mol_type = other DNA
gacattgtgatgacccagagccccgactccctggccgtgagcctgggagaaagagccaccatcaactgcaagagcagccagagcgtgctgagcagcggcaaccagaaaaactacctggcctggtaccagcagaagcccggccagccccccaagctgctgatctactgggccagcaccagagagagcggcgtgcccgacagattcagcggcagcggcagcggcaccgacttcaccctgaccatcagcagcctgcaggccgaggacgtggccgtgtactactgccagaacgcctactactaccccttcaccttcggccagggcaccaagctggagatcaagcgtacggtggctgcaccatctgtcttcatcttcccgccatctgatgagcagttgaaatctggaactgcctctgttgtgtgcctgctgaataacttctatcccagagaggccaaagtacagtggaaggtggataacgccctccaatcgggtaactcccaggagagtgtcacagagcaggacagcaaggacagcacctacagcctcagcagcaccctgacgctgagcaaagcagactacgagaaacacaaagtctacgcctgcgaagtcacccatcagggcctgagttcgcccgtcacaaagagcttcaacaggggagagtgt

SEQ ID NO: 25 - protein, 125 aa, synthetic construct
QVQLVESGGGVVQPGRSLRLSCAASGSTFSIVAMGWYRQAPGKQRELVASIITGDGDTNYADSVKGRFTISRDNSKNTMYLQMNSLKPEDTAVYYCYARTGYGSSELEGHEYDYWGQGTQVTVSS

SEQ ID NO: 26 - protein, 21 aa, synthetic construct
GGGGSGGGGSGGGGSGGGGSG

SEQ ID NO: 27 - protein, 595 aa, synthetic construct
QVQLVQSGAEVKKPGASVKVSCKASGYTFTSYYMHWVRQAPGQGLEWMGTIYPGNGDTSYNQKFQGRVTMTRDKSTSTVYMELSSLRSEDTAVYFCARGGYYGNSLDYWGQGTLVTVSSASTKGPSVFPLAPSSKSTSGGTAALGCLVKDYFPEPVTVSWNSGALTSGVHTFPAVLQSSGLYSLSSVVTVPSSSLGTQTYICNVNHKPSNTKVDKKVEPKSCDKTHTCPPCPAPEAAGGPSVFLFPPKPKDTLMISRTPEVTCVVVDVSHEDPEVKFNWYVDGVEVHNAKTKPREEQYNSTYRVVSVLTVLHQDWLNGKEYKCKVSNKALPAPIEKTISKAKGQPREPQVYTLPPSREEMTKNQVSLTCLVKGFYPSDIAVEWESNGQPENNYKTTPPVLDSDGSFFLYSKLTVDKSRWQQGNVFSCSVMHEALHNHYTQKSLSLSPGKGGGGSGGGGSGGGGSGGGGSGQVQLVESGGGVVQPGRSLRLSCAASGSTFSIVAMGWYRQAPGKQRELVASIITGDGDTNYADSVKGRFTISRDNSKNTMYLQMNSLKPEDTAVYYCYARTGEGSSWLEGHEYDYWGQGTQVTVSS

SEQ ID NO: 28 - protein, 595 aa, synthetic construct
QVQLVQSGAEVKKPGASVKVSCKASGYTFTSYYMHWVRQAPGQGLEWMGTIYPGNGDTSYNQKFQGRVTMTRDKSTSTVYMELSSLRSEDTAVYFCARGGYYGNSLDYWGQGTLVTVSSASTKGPSVFPLAPSSKSTSGGTAALGCLVKDYFPEPVTVSWNSGALTSGVHTFPAVLQSSGLYSLSSVVTVPSSSLGTQTYICNVNHKPSNTKVDKKVEPKSCDKTHTCPPCPAPEAAGGPSVFLFPPKPKDTLMISRTPEVTCVVVDVSHEDPEVKFNWYVDGVEVHNAKTKPREEQYNSTYRVVSVLTVLHQDWLNGKEYKCKVSNKALPAPIEKTISKAKGQPREPQVYTLPPSREEMTKNQVSLTCLVKGFYPSDIAVEWESNGQPENNYKTTPPVLDSDGSFFLYSKLTVDKSRWQQGNVFSCSVMHEALHNHYTQKSLSLSPGKGGGGSGGGGSGGGGSGGGGSGQVQLVESGGGVVQPGRSLRLSCAASGSTFSIVAMGWYRQAPGKQRELVASIITGDGDTNYADSVKGRFTISRDNSKNTMYLQMNSLKPEDTAVYYCYARTGYGSSELEGHEYDYWGQGTQVTVSS

SEQ ID NO: 29 - protein, 594 aa, synthetic construct
QVQLVQSGAEVKKPGASVKVSCKASGYTFTSYYMHWVRQAPGQGLEWMGTIYPGNGDTSYNQKFQGRVTMTRDKSTSTVYMELSSLRSEDTAVYFCARGGYYGNSLDYWGQGTLVTVSSASTKGPSVFPLAPSSKSTSGGTAALGCLVKDYFPEPVTVSWNSGALTSGVHTFPAVLQSSGLYSLSSVVTVPSSSLGTQTYICNVNHKPSNTKVDKKVEPKSCDKTHTCPPCPAPEAAGGPSVFLFPPKPKDTLMISRTPEVTCVVVDVSHEDPEVKFNWYVDGVEVHNAKTKPREEQYNSTYRVVSVLTVLHQDWLNGKEYKCKVSNKALPAPIEKTISKAKGQPREPQVYTLPPSREEMTKNQVSLTCLVKGFYPSDIAVEWESNGQPENNYKTTPPVLDSDGSFFLYSKLTVDKSRWQQGNVFSCSVMHEALHNHYTQKSLSLSPGKGGGGSGGGGSGGGGSGGGGSQVQLVESGGGVVQPGRSLRLSCAASGSTFSIVAMGWYRQAPGKQRELVASIITGDGDTNYADSVKGRFTISRDNSKNTMYLQMNSLKPEDTAVYYCYARTGYGSSELEGHEYDYWGQGTQVTVSS